European Patent Application EP 4 119 143 A1, published January 18, 2023. Title: Pharmaceutical composition for preventing or treating NK-T cell lymphoma or NK cell leukemia, comprising phosphodiesterase 5 inhibitor. Applicant: SAMSUNG LIFE PUBLIC WELFARE FOUNDATION. The sequence listing filed with the application follows.

SEQUENCE LISTING (8 sequences)

SEQ ID NO: 1 - DNA, 24 bp, Artificial Sequence
  BZLF1-Forward primer
aatgccgggccaagtttaagcaac

SEQ ID NO: 2 - DNA, 24 bp, Artificial Sequence
  BZLF1-reverse primer
ttgggcacatctgcttcaacagga

SEQ ID NO: 3 - DNA, 24 bp, Artificial Sequence
  BRLF1-Forward primer
tggcttggaagactttctgaggct

SEQ ID NO: 4 - DNA, 24 bp, Artificial Sequence
  BRLF1-reverse primer
aatctccacactcccggctgtaaa

SEQ ID NO: 5 - DNA, 21 bp, Artificial Sequence
  GAPDH-Forward primer
ggcatggactgtggtcatgag

SEQ ID NO: 6 - DNA, 20 bp, Artificial Sequence
  GAPDH-reverse primer
tgcaccaccaactgcttagc

SEQ ID NO: 7 - DNA, 21 bp, Artificial Sequence
  BALF5-Forward primer
cgtctcattcccaagtgtttc

SEQ ID NO: 8 - DNA, 18 bp, Artificial Sequence
  BALF5-Reverse primer
gccctttccatcctcgtc